European Patent Application EP 4 317 175 A1, published February 7, 2024. Title: TRUNCATED TACI POLYPEPTIDE AND FUSION PROTEIN AND USE THEREOF. Applicant: JIANGSU HENGRUI PHARMACEUTICALS CO., LTD. SHANGHAI HENGRUI PHARMACEUTICAL CO., LTD. Application PCT/CN2022/084256. The sequence listing filed with the application follows.

SEQUENCE LISTING (73 sequences)

SEQ ID NO: 1 - protein, 165 aa, Homo sapiens
MSGLGRSRRGGRSRVDQEERFPQGLWTGVAMRSCPEEQYWDPLLGTCMSCKTICNHQSQRTCAAFCRSLSCRKEQGKFYDHLLRDCISCASICGQHPKQCAYFCENKLRSPVNLPPELRRQRSGEVENNSDNSGRYQGLEHRGSEASPALPGLKLSADQVALVYS

SEQ ID NO: 2 - protein, 164 aa, Artificial Sequence
  TACI-1
SGLGRSRKGGKSRVDQEERFPQGLWTGVAMRSCPEEQYWDPLLGTCMSCKTICNHQSQRTCAAFCRSLSCRKEQGKFYDHLLRDCISCASICGQHPKQCAYFCENKLRSPVNLPPELRKQRSGEVEQNSDNSGKYQGLEHRGSEASPALPGLKLSADQVALVYS

SEQ ID NO: 3 - protein, 133 aa, Artificial Sequence
  TACI-2
SGLGRSRKGGKSRVDQEERFPQGLWTGVAMRSCPEEQYWDPLLGTCMSCKTICNHQSQRTCAAFCRSLSCRKEQGKFYDHLLRDCISCASICGQHPKQCAYFCENKLRSPVNLPPELRKQRSGEVENNSDNSG

SEQ ID NO: 4 - protein, 126 aa, Artificial Sequence
  TACI-3
SGLGRSRKGGKSRVDQEERFPQGLWTGVAMRSCPEEQYWDPLLGTCMSCKTICNHQSQRTCAAFCRSLSCRKEQGKFYDHLLRDCISCASICGQHPKQCAYFCENKLRSPVNLPPELRKQRSGEVE

SEQ ID NO: 5 - protein, 156 aa, Artificial Sequence
  TACI-4
GGRSRVDQEERFPQGLWTGVAMRSCPEEQYWDPLLGTCMSCKTICNHQSQRTCAAFCRSLSCRKEQGKFYDHLLRDCISCASICGQHPKQCAYFCENKLRSPVNLPPELRKQRSGEVENNSDNSGKYQGLEHRGSEASPALPGLKLSADQVALVYS

SEQ ID NO: 6 - protein, 125 aa, Artificial Sequence
  TACI-5
GGRSRVDQEERFPQGLWTGVAMRSCPEEQYWDPLLGTCMSCKTICNHQSQRTCAAFCRSLSCRKEQGKFYDHLLRDCISCASICGQHPKQCAYFCENKLRSPVNLPPELRKQRSGEVENNSDNSG

SEQ ID NO: 7 - protein, 118 aa, Artificial Sequence
  TACI-6
GGRSRVDQEERFPQGLWTGVAMRSCPEEQYWDPLLGTCMSCKTICNHQSQRTCAAFCRSLSCRKEQGKFYDHLLRDCISCASICGQHPKQCAYFCENKLRSPVNLPPELRKQRSGEVE

SEQ ID NO: 8 - protein, 96 aa, Artificial Sequence
  TACI-7
FPQGLWTGVAMRSCPEEQYWDPLLGTCMSCKTICNHQSQRTCAAFCRSLSCRKEQGKFYDHLLRDCISCASICGQHPKQCAYFCENKLRSPVNLPP

SEQ ID NO: 9 - protein, 98 aa, Artificial Sequence
  TACI-8
SLSCRKEQGKFYDHLLRDCISCASICGQHPKQCAYFCENKLRSPVNLPPELRKQRSGEVENNSDNSGKYQGLEHRGSEASPALPGLKLSADQVALVYS

SEQ ID NO: 10 - protein, 41 aa, Artificial Sequence
  TACI-9
SLSCRKEQGKFYDHLLRDCISCASICGQHPKQCAYFCENKL

SEQ ID NO: 11 - protein, 227 aa, Homo sapiens
DKTHTCPPCPAPEAEGAPSVFLFPPKPKDTLMISRTPEVTCVVVDVSHEDPEVKFNWYVDGVEVHNAKTKPREEQYNSTYRVVSVLTVLHQDWLNGKEYKCKVSNKALPSSIEKTISKAKGQPREPQVYTLPPSRDELTKNQVSLTCLVKGFYPSDIAVEWESNGQPENNYKTTPPVLDSDGSFFLYSKLTVDKSRWQQGNVFSCSVMHEALHNHYTQKSLSLSPGK

SEQ ID NO: 12 - protein, 333 aa, Artificial Sequence
  Amino acid sequence of RCT-18
SRVDQEERFPQGLWTGVAMRSCPEEQYWDPLLGTCMSCKTICNHQSQRTCAAFCRSLSCRKEQGKFYDHLLRDCISCASICGQHPKQCAYFCENKLRSPVNLPPELDKTHTCPPCPAPEAEGAPSVFLFPPKPKDTLMISRTPEVTCVVVDVSHEDPEVKFNWYVDGVEVHNAKTKPREEQYNSTYRVVSVLTVLHQDWLNGKEYKCKVSNKALPSSIEKTISKAKGQPREPQVYTLPPSRDELTKNQVSLTCLVKGFYPSDIAVEWESNGQPENNYKTTPPVLDSDGSFFLYSKLTVDKSRWQQGNVFSCSVMHEALHNHYTQKSLSLSPGK

SEQ ID NO: 13 - protein, 40 aa, Artificial Sequence
  TACI-10
SLSCRKEQGKFYDHLLRDCISCASICGQHPKQCAYFCENK

SEQ ID NO: 14 - protein, 39 aa, Artificial Sequence
  TACI-11
SLSCRKEQGKFYDHLLRDCISCASICGQHPKQCAYFCEN

SEQ ID NO: 15 - protein, 38 aa, Artificial Sequence
  TACI-12
SLSCRKEQGKFYDHLLRDCISCASICGQHPKQCAYFCE

SEQ ID NO: 16 - protein, 37 aa, Artificial Sequence
  TACI-13
SLSCRKEQGKFYDHLLRDCISCASICGQHPKQCAYFC

SEQ ID NO: 17 - protein, 36 aa, Artificial Sequence
  TACI-14
SLSCRKEQGKFYDHLLRDCISCASICGQHPKQCAYF

SEQ ID NO: 18 - protein, 41 aa, Artificial Sequence
  TACI-9-1
STSCRKEQGKFYDHLLRDCISCASICGQHPKQCAYFCENKL

SEQ ID NO: 19 - protein, 41 aa, Artificial Sequence
  TACI-9-2
SLSCSKEQGKFYDHLLRDCISCASICGQHPKQCAYFCENKL

SEQ ID NO: 20 - protein, 41 aa, Artificial Sequence
  TACI-9-3
SLSCREEQGKFYDHLLRDCISCASICGQHPKQCAYFCENKL

SEQ ID NO: 21 - protein, 41 aa, Artificial Sequence
  TACI-9-4
SLSCRQEQGKFYDHLLRDCISCASICGQHPKQCAYFCENKL

SEQ ID NO: 22 - protein, 41 aa, Artificial Sequence
  TACI-9-5
SLSCRKEQGEFYDHLLRDCISCASICGQHPKQCAYFCENKL

SEQ ID NO: 23 - protein, 41 aa, Artificial Sequence
  TACI-9-6
SRSCRKEQGKFYDHLLRTCISCASICGQHPKQCAYFCENKL

SEQ ID NO: 24 - protein, 41 aa, Artificial Sequence
  TACI-9-7
SRSCRKEQGKFYDHLLRACISCASICGQHPKQCAYFCENKL

SEQ ID NO: 25 - protein, 41 aa, Artificial Sequence
  TACI-9-8
SLSCRKEQGKFYDHLLRDCISCASICGQHPKQCAAFCENKL

SEQ ID NO: 26 - protein, 41 aa, Artificial Sequence
  TACI-9-9
SRSCRKEQGKFYDHLLRTCISCASICGQHPKQCARFCENKL

SEQ ID NO: 27 - protein, 41 aa, Artificial Sequence
  TACI-9-10
SLSCREEQGEFYDHLLRDCISCASICGQHPKQCAYFCENKL

SEQ ID NO: 28 - protein, 41 aa, Artificial Sequence
  TACI-9-11
SLSCSEEQGEFYDHLLRDCISCASICGQHPKQCAYFCENKL

SEQ ID NO: 29 - protein, 41 aa, Artificial Sequence
  TACI-9-12
STSCRKEQGKFYDHLLRDCISCASICGQHPKQCAAFCENKL

SEQ ID NO: 30 - protein, 41 aa, Artificial Sequence
  TACI-9-13
STSCRKEQGKFYDHLLRDCISCASICGQHPKQCAYYCENKL

SEQ ID NO: 31 - protein, 41 aa, Artificial Sequence
  TACI-9-14
STSCRKEQGKFYDHLLRDCISCASICGQHPKQCAAYCENKL

SEQ ID NO: 32 - protein, 41 aa, Artificial Sequence
  TACI-9-15
STSCREEQGEFYDHLLRDCISCASICGQHPKQCAAFCENKL

SEQ ID NO: 33 - protein, 40 aa, Artificial Sequence
  TACI-9-15a
STSCREEQGEFYDHLLRDCISCASICGQHPKQCAAFCENK

SEQ ID NO: 34 - protein, 39 aa, Artificial Sequence
  TACI-9-15b
STSCREEQGEFYDHLLRDCISCASICGQHPKQCAAFCEN

SEQ ID NO: 35 - protein, 38 aa, Artificial Sequence
  TACI-9-15c
STSCREEQGEFYDHLLRDCISCASICGQHPKQCAAFCE

SEQ ID NO: 36 - protein, 273 aa, Artificial Sequence
  Sequence of TACI-9-15Fc1 fusion protein
STSCREEQGEFYDHLLRDCISCASICGQHPKQCAAFCENKLEPKSSDKTHTCPPCPAPELLGGPSVFLFPPKPKDTLMISRTPEVTCVVVDVSHEDPEVKFNWYVDGVEVHNAKTKPREEQYNSTYRVVSVLTVLHQDWLNGKEYKCKVSNKALPAPIEKTISKAKGQPREPQVYTLPPSRDELTKNQVSLTCLVKGFYPSDIAVEWESNGQPENNYKTTPPVLDSDGSFFLYSKLTVDKSRWQQGNVFSCSVMHEALHNHYTQKSLSLSPGK

SEQ ID NO: 37 - protein, 271 aa, Artificial Sequence
  Sequence of TACI-9-15Fc2 fusion protein
STSCREEQGEFYDHLLRDCISCASICGQHPKQCAAFCENEPKSSDKTHTCPPCPAPELLGGPSVFLFPPKPKDTLMISRTPEVTCVVVDVSHEDPEVKFNWYVDGVEVHNAKTKPREEQYNSTYRVVSVLTVLHQDWLNGKEYKCKVSNKALPAPIEKTISKAKGQPREPQVYTLPPSRDELTKNQVSLTCLVKGFYPSDIAVEWESNGQPENNYKTTPPVLDSDGSFFLYSKLTVDKSRWQQGNVFSCSVMHEALHNHYTQKSLSLSPGK

SEQ ID NO: 38 - protein, 270 aa, Artificial Sequence
  Sequence of TACI-9-15Fc3 fusion protein
STSCREEQGEFYDHLLRDCISCASICGQHPKQCAAFCEEPKSSDKTHTCPPCPAPELLGGPSVFLFPPKPKDTLMISRTPEVTCVVVDVSHEDPEVKFNWYVDGVEVHNAKTKPREEQYNSTYRVVSVLTVLHQDWLNGKEYKCKVSNKALPAPIEKTISKAKGQPREPQVYTLPPSRDELTKNQVSLTCLVKGFYPSDIAVEWESNGQPENNYKTTPPVLDSDGSFFLYSKLTVDKSRWQQGNVFSCSVMHEALHNHYTQKSLSLSPGK

SEQ ID NO: 39 - protein, 270 aa, Artificial Sequence
  Sequence of TACI-9-15Fc4 fusion protein
DKTHTCPPCPAPELLGGPSVFLFPPKPKDTLMISRTPEVTCVVVDVSHEDPEVKFNWYVDGVEVHNAKTKPREEQYNSTYRVVSVLTVLHQDWLNGKEYKCKVSNKALPAPIEKTISKAKGQPREPQVYTLPPSRDELTKNQVSLTCLVKGFYPSDIAVEWESNGQPENNYKTTPPVLDSDGSFFLYSKLTVDKSRWQQGNVFSCSVMHEALHNHYTQKSLSLSPGGGGSSTSCREEQGEFYDHLLRDCISCASICGQHPKQCAAFCENK

SEQ ID NO: 40 - protein, 265 aa, Artificial Sequence
  Sequence of TACI-9-15Fc5 fusion protein
STSCREEQGEFYDHLLRDCISCASICGQHPKQCAAFCEDKTHTCPPCPAPEAEGAPSVFLFPPKPKDTLMISRTPEVTCVVVDVSHEDPEVKFNWYVDGVEVHNAKTKPREEQYNSTYRVVSVLTVLHQDWLNGKEYKCKVSNKALPSSIEKTISKAKGQPREPQVYTLPPSRDELTKNQVSLTCLVKGFYPSDIAVEWESNGQPENNYKTTPPVLDSDGSFFLYSKLTVDKSRWQQGNVFSCSVMHEALHNHYTQKSLSLSPGK

SEQ ID NO: 41 - protein, 270 aa, Artificial Sequence
  Sequence of TACI-9-15Fc6 fusion protein
STSCREEQGEFYDHLLRDCISCASICGQHPKQCAAFCEEPKSSDKTHTCPPCPAPEAEGAPSVFLFPPKPKDTLMISRTPEVTCVVVDVSHEDPEVKFNWYVDGVEVHNAKTKPREEQYNSTYRVVSVLTVLHQDWLNGKEYKCKVSNKALPSSIEKTISKAKGQPREPQVYTLPPSRDELTKNQVSLTCLVKGFYPSDIAVEWESNGQPENNYKTTPPVLDSDGSFFLYSKLTVDKSRWQQGNVFSCSVMHEALHNHYTQKSLSLSPGK

SEQ ID NO: 42 - protein, 313 aa, Artificial Sequence
  Sequence of TACI-9-15Fc7 fusion protein
STSCREEQGEFYDHLLRDCISCASICGQHPKQCAAFCEEPKSSDKTHTCPPCPAPEAEGAPSVFLFPPKPKDTLMISRTPEVTCVVVDVSHEDPEVKFNWYVDGVEVHNAKTKPREEQYNSTYRVVSVLTVLHQDWLNGKEYKCKVSNKALPSSIEKTISKAKGQPREPQVYTLPPSRDELTKNQVSLTCLVKGFYPSDIAVEWESNGQPENNYKTTPPVLDSDGSFFLYSKLTVDKSRWQQGNVFSCSVMHEALHNHYTQKSLSLSPGGGGSSTSCREEQGEFYDHLLRDCISCASICGQHPKQCAAFCEQK

SEQ ID NO: 43 - protein, 313 aa, Artificial Sequence
  Sequence of TACI-9-15Fc8 fusion protein
STSCREEQGEFYDHLLRDCISCASICGQHPKQCAAFCEEPKSSDKTHTCPPCPAPEAEGAPSVFLFPPKPKDTLMISRTPEVTCVVVDVSHEDPEVKFNWYVDGVEVHNAKTKPREEQYNSTYRVVSVLTVLHQDWLNGKEYKCKVSNKALPSSIEKTISKAKGQPREPQVYTLPPSRDELTKNQVSLTCLVKGFYPSDIAVEWESNGQPENNYKTTPPVLDSDGSFFLYSKLTVDKSRWQQGNVFSCSVMHEALHNHYTQKSLSLSPGGGGSSTSCREEQGEFYDHLLRDCISCASICGQHPKQCAAFCESK

SEQ ID NO: 44 - protein, 313 aa, Artificial Sequence
  Sequence of TACI-9-15Fc9 fusion protein
STSCREEQGEFYDHLLRDCISCASICGQHPKQCAAFCEEPKSSDKTHTCPPCPAPEAEGAPSVFLFPPKPKDTLMISRTPEVTCVVVDVSHEDPEVKFNWYVDGVEVHNAKTKPREEQYNSTYRVVSVLTVLHQDWLNGKEYKCKVSNKALPSSIEKTISKAKGQPREPQVYTLPPSRDELTKNQVSLTCLVKGFYPSDIAVEWESNGQPENNYKTTPPVLDSDGSFFLYSKLTVDKSRWQQGNVFSCSVMHEALHNHYTQKSLSLSPGGGGSSTSCREEQGEFYDHLLRDCISCASICGQHPKQCAAFCESS

SEQ ID NO: 45 - protein, 119 aa, Artificial Sequence
  Heavy chain variable region of ustekinumab
EVQLVQSGAEVKKPGESLKISCKGSGYSFTTYWLGWVRQMPGKGLDWIGIMSPVDSDIRYSPSFQGQVTMSVDKSITTAYLQWNSLKASDTAMYYCARRRPGQGYFDFWGQGTLVTVSS

SEQ ID NO: 46 - protein, 107 aa, Artificial Sequence
  Light chain variable region of ustekinumab
DIQMTQSPSSLSASVGDRVTITCRASQGISSWLAWYQQKPEKAPKSLIYAASSLQSGVPSRFSGSGSGTDFTLTISSLQPEDFATYYCQQYNIYPYTFGQGTKLEIK

SEQ ID NO: 47 - protein, 449 aa, Artificial Sequence
  Heavy chain of ustekinumab
EVQLVQSGAEVKKPGESLKISCKGSGYSFTTYWLGWVRQMPGKGLDWIGIMSPVDSDIRYSPSFQGQVTMSVDKSITTAYLQWNSLKASDTAMYYCARRRPGQGYFDFWGQGTLVTVSSSSTKGPSVFPLAPSSKSTSGGTAALGCLVKDYFPEPVTVSWNSGALTSGVHTFPAVLQSSGLYSLSSVVTVPSSSLGTQTYICNVNHKPSNTKVDKRVEPKSCDKTHTCPPCPAPELLGGPSVFLFPPKPKDTLMISRTPEVTCVVVDVSHEDPEVKFNWYVDGVEVHNAKTKPREEQYNSTYRVVSVLTVLHQDWLNGKEYKCKVSNKALPAPIEKTISKAKGQPREPQVYTLPPSRDELTKNQVSLTCLVKGFYPSDIAVEWESNGQPENNYKTTPPVLDSDGSFFLYSKLTVDKSRWQQGNVFSCSVMHEALHNHYTQKSLSLSPGK

SEQ ID NO: 48 - protein, 214 aa, Artificial Sequence
  Light chain of ustekinumab
DIQMTQSPSSLSASVGDRVTITCRASQGISSWLAWYQQKPEKAPKSLIYAASSLQSGVPSRFSGSGSGTDFTLTISSLQPEDFATYYCQQYNIYPYTFGQGTKLEIKRTVAAPSVFIFPPSDEQLKSGTASVVCLLNNFYPREAKVQWKVDNALQSGNSQESVTEQDSKDSTYSLSSTLTLSKADYEKHKVYACEVTHQGLSSPVTKSFNRGEC

SEQ ID NO: 49 - protein, 11 aa, Artificial Sequence
  Ustekinumab LCDR1
RASQGISSWLA

SEQ ID NO: 50 - protein, 7 aa, Artificial Sequence
  Ustekinumab LCDR2
AASSLQS

SEQ ID NO: 51 - protein, 9 aa, Artificial Sequence
  Ustekinumab LCDR3
QQYNIYPYT

SEQ ID NO: 52 - protein, 5 aa, Artificial Sequence
  Ustekinumab HCDR1
TYWLG

SEQ ID NO: 53 - protein, 17 aa, Artificial Sequence
  Ustekinumab HCDR2
IMSPVDSDIRYSPSFQG

SEQ ID NO: 54 - protein, 10 aa, Artificial Sequence
  Ustekinumab HCDR3
RRPGQGYFDF

SEQ ID NO: 55 - protein, 492 aa, Artificial Sequence
  Heavy chain of TACI-Mab1
EVQLVQSGAEVKKPGESLKISCKGSGYSFTTYWLGWVRQMPGKGLDWIGIMSPVDSDIRYSPSFQGQVTMSVDKSITTAYLQWNSLKASDTAMYYCARRRPGQGYFDFWGQGTLVTVSSASTKGPSVFPLAPSSKSTSGGTAALGCLVKDYFPEPVTVSWNSGALTSGVHTFPAVLQSSGLYSLSSVVTVPSSSLGTQTYICNVNHKPSNTKVDKKVEPKSCDKTHTCPPCPAPELLGGPSVFLFPPKPKDTLMISRTPEVTCVVVDVSHEDPEVKFNWYVDGVEVHNAKTKPREEQYNSTYRVVSVLTVLHQDWLNGKEYKCKVSNKALPAPIEKTISKAKGQPREPQVYTLPPSRDELTKNQVSLTCLVKGFYPSDIAVEWESNGQPENNYKTTPPVLDSDGSFFLYSKLTVDKSRWQQGNVFSCSVMHEALHNHYTQKSLSLSPGGGGSSTSCREEQGEFYDHLLRDCISCASICGQHPKQCAAFCENK

SEQ ID NO: 56 - protein, 214 aa, Artificial Sequence; identical to SEQ ID NO: 48
  Light chain of TACI-Mab1

SEQ ID NO: 57 - protein, 492 aa, Artificial Sequence; identical to SEQ ID NO: 55
  Heavy chain of TACI-Mab2

SEQ ID NO: 58 - protein, 270 aa, Artificial Sequence
  Light chain of TACI-Mab2
STSCREEQGEFYDHLLRDCISCASICGQHPKQCAAFCENKLGGGGSGGGGSGGGGSDIQMTQSPSSLSASVGDRVTITCRASQGISSWLAWYQQKPEKAPKSLIYAASSLQSGVPSRFSGSGSGTDFTLTISSLQPEDFATYYCQQYNIYPYTFGQGTKLEIKRTVAAPSVFIFPPSDEQLKSGTASVVCLLNNFYPREAKVQWKVDNALQSGNSQESVTEQDSKDSTYSLSSTLTLSKADYEKHKVYACEVTHQGLSSPVTKSFNRGEC

SEQ ID NO: 59 - protein, 453 aa, Artificial Sequence
  Heavy chain of belimumab
QVQLQQSGAEVKKPGSSVRVSCKASGGTFNNNAINWVRQAPGQGLEWMGGIIPMFGTAKYSQNFQGRVAITADESTGTASMELSSLRSEDTAVYYCARSRDLLLFPHHALSPWGRGTMVTVSSASTKGPSVFPLAPSSKSTSGGTAALGCLVKDYFPEPVTVSWNSGALTSGVHTFPAVLQSSGLYSLSSVVTVPSSSLGTQTYICNVNHKPSNTKVDKKVEPKSCDKTHTCPPCPAPELLGGPSVFLFPPKPKDTLMISRTPEVTCVVVDVSHEDPEVKFNWYVDGVEVHNAKTKPREEQYNSTYRVVSVLTVLHQDWLNGKEYKCKVSNKALPAPIEKTISKAKGQPREPQVYTLPPSRDELTKNQVSLTCLVKGFYPSDIAVEWESNGQPENNYKTTPPVLDSDGSFFLYSKLTVDKSRWQQGNVFSCSVMHEALHNHYTQKSLSLSPGK

SEQ ID NO: 60 - protein, 214 aa, Artificial Sequence
  Light chain of belimumab
SSELTQDPAVSVALGQTVRVTCQGDSLRSYYASWYQQKPGQAPVLVIYGKNNRPSGIPDRFSGSSSGNTASLTITGAQAEDEADYYCSSRDSSGNHWVFGGGTELTVLGQPKAAPSVTLFPPSSEELQANKATLVCLISDFYPGAVTVAWKADSSPVKAGVETTTPSKQSNNKYAASSYLSLTPEQWKSHRSYSCQVTHEGSTVEKTVAPTECS

SEQ ID NO: 61 - protein, 227 aa, Artificial Sequence
  Fc sequence 1 of human IgG
DKTHTCPPCPAPELLGGPSVFLFPPKPKDTLMISRTPEVTCVVVDVSHEDPEVKFNWYVDGVEVHNAKTKPREEQYNSTYRVVSVLTVLHQDWLNGKEYKCKVSNKALPAPIEKTISKAKGQPREPQVYTLPPSRDELTKNQVSLTCLVKGFYPSDIAVEWESNGQPENNYKTTPPVLDSDGSFFLYSKLTVDKSRWQQGNVFSCSVMHEALHNHYTQKSLSLSPGK

SEQ ID NO: 62 - protein, 226 aa, Artificial Sequence
  Fc sequence 2 of human IgG
DKTHTCPPCPAPELLGGPSVFLFPPKPKDTLMISRTPEVTCVVVDVSHEDPEVKFNWYVDGVEVHNAKTKPREEQYNSTYRVVSVLTVLHQDWLNGKEYKCKVSNKALPAPIEKTISKAKGQPREPQVYTLPPSRDELTKNQVSLTCLVKGFYPSDIAVEWESNGQPENNYKTTPPVLDSDGSFFLYSKLTVDKSRWQQGNVFSCSVMHEALHNHYTQKSLSLSPG

SEQ ID NO: 63 - protein, 226 aa, Artificial Sequence
  Fc sequence 3 of human IgG
DKTHTCPPCPAPEAEGAPSVFLFPPKPKDTLMISRTPEVTCVVVDVSHEDPEVKFNWYVDGVEVHNAKTKPREEQYNSTYRVVSVLTVLHQDWLNGKEYKCKVSNKALPSSIEKTISKAKGQPREPQVYTLPPSRDELTKNQVSLTCLVKGFYPSDIAVEWESNGQPENNYKTTPPVLDSDGSFFLYSKLTVDKSRWQQGNVFSCSVMHEALHNHYTQKSLSLSPG

SEQ ID NO: 64 - protein, 5 aa, Artificial Sequence
  Linker sequence 1
EPKSS

SEQ ID NO: 65 - protein, 4 aa, Artificial Sequence
  Linker sequence 2
GGGS

SEQ ID NO: 66 - protein, 5 aa, Artificial Sequence
  Linker sequence 3
GGGGS

SEQ ID NO: 67 - protein, 15 aa, Artificial Sequence
  Linker sequence 4
GGGGSGGGGSGGGGS

SEQ ID NO: 68 - protein, 37 aa, Artificial Sequence
  TACI-16
LSCRKEQGKFYDHLLRDCISCASICGQHPKQCAYFCE

SEQ ID NO: 69 - protein, 36 aa, Artificial Sequence
  TACI-17
SCRKEQGKFYDHLLRDCISCASICGQHPKQCAYFCE

SEQ ID NO: 70 - protein, 35 aa, Artificial Sequence
  TACI-18
CRKEQGKFYDHLLRDCISCASICGQHPKQCAYFCE

SEQ ID NO: 71 - protein, 34 aa, Artificial Sequence
  TACI-19
RKEQGKFYDHLLRDCISCASICGQHPKQCAYFCE

SEQ ID NO: 72 - protein, 33 aa, Artificial Sequence
  TACI-20
KEQGKFYDHLLRDCISCASICGQHPKQCAYFCE

SEQ ID NO: 73 - protein, 32 aa, Artificial Sequence
  TACI-21
EQGKFYDHLLRDCISCASICGQHPKQCAYFCE